European Patent Application EP 4 410 296 A1, published August 7, 2024. Title: 直接转分化治疗神经系统疾病. Applicant: 中国科学院脑科学与智能技术卓越创新中心. The sequence listing filed with the application follows.

SEQUENCE LISTING (58 sequences)

SEQ ID NO: 1 - protein, 266 aa, Homo sapiens
KTKPFRCKPCQYEAESEEQFVHHIRVHSAKKFFVEESAEKQAKARESGSSTAEEGDFSKGPIRCDRCGYNTNRYDHYTAHLKHHTRAGDNERVYKCIICTYTTVSEYHWRKHLRNHFPRKVYTCGKCNYFSDRKNNYVQHVRTHTGERPYKCELCPYSSSQKTHLTRHMRTHSGEKPFKCDQCSYVASNQHEVTRHARQVHNGPKPLNCPHCDYKTADRSNFKKHVELHVNPRQFNCPVCDYAASKKCNLQYHFKSKHPTCPNKTM

SEQ ID NO: 2 - DNA, 798 bp, Homo sapiens
  source 1..798: mol_type = genomic DNA
aagaccaaaccctttcgctgtaagccatgccaatatgaagcagaatctgaagaacagtttgtgcatcacatcagagttcacagtgctaagaaattttttgtggaagagagtgcagagaagcaggcaaaagccagggaatctggctcttccactgcagaagagggagatttctccaagggccccattcgctgtgaccgctgcggctacaatactaatcgatatgatcactatacagcacacctgaaacaccacaccagagctggggataatgagcgagtctacaagtgtatcatttgcacatacacaacagtgagcgagtatcactggaggaaacatttaagaaaccattttccaaggaaagtatacacatgtggaaaatgcaactatttttcagacagaaaaaacaattatgttcagcatgttagaactcatacaggagaacgcccatataaatgtgaactttgtccttactcaagttctcagaagactcatctaactagacatatgcgtactcattcaggtgagaagccatttaaatgtgatcagtgcagttatgtggcctctaatcaacatgaagtaacccgccatgcaagacaggttcacaatgggcctaaacctcttaattgcccacactgtgattacaaaacagcagatagaagcaacttcaaaaaacatgtagagctacatgtgaacccacggcagttcaattgccctgtatgtgactatgcagcttccaagaagtgtaatctacagtatcacttcaaatctaagcatcctacttgtcctaataaaacaatg

SEQ ID NO: 3 - protein, 277 aa, Artificial Sequence
MPKKKRKVGSGKTKPFRCKPCQYEAESEEQFVHHIRVHSAKKFFVEESAEKQAKARESGSSTAEEGDFSKGPIRCDRCGYNTNRYDHYTAHLKHHTRAGDNERVYKCIICTYTTVSEYHWRKHLRNHFPRKVYTCGKCNYFSDRKNNYVQHVRTHTGERPYKCELCPYSSSQKTHLTRHMRTHSGEKPFKCDQCSYVASNQHEVTRHARQVHNGPKPLNCPHCDYKTADRSNFKKHVELHVNPRQFNCPVCDYAASKKCNLQYHFKSKHPTCPNKTM

SEQ ID NO: 4 - DNA, 831 bp, Artificial Sequence
  source 1..831: mol_type = other DNA
atgcctaaaaagaaaagaaaggtgggttctggtaagaccaaaccctttcgctgtaagccatgccaatatgaagcagaatctgaagaacagtttgtgcatcacatcagagttcacagtgctaagaaattttttgtggaagagagtgcagagaagcaggcaaaagccagggaatctggctcttccactgcagaagagggagatttctccaagggccccattcgctgtgaccgctgcggctacaatactaatcgatatgatcactatacagcacacctgaaacaccacaccagagctggggataatgagcgagtctacaagtgtatcatttgcacatacacaacagtgagcgagtatcactggaggaaacatttaagaaaccattttccaaggaaagtatacacatgtggaaaatgcaactatttttcagacagaaaaaacaattatgttcagcatgttagaactcatacaggagaacgcccatataaatgtgaactttgtccttactcaagttctcagaagactcatctaactagacatatgcgtactcattcaggtgagaagccatttaaatgtgatcagtgcagttatgtggcctctaatcaacatgaagtaacccgccatgcaagacaggttcacaatgggcctaaacctcttaattgcccacactgtgattacaaaacagcagatagaagcaacttcaaaaaacatgtagagctacatgtgaacccacggcagttcaattgccctgtatgtgactatgcagcttccaagaagtgtaatctacagtatcacttcaaatctaagcatcctacttgtcctaataaaacaatg

SEQ ID NO: 5 - protein, 344 aa, Artificial Sequence
MPKKKRKVGSGKTKPFRCKPCQYEAESEEQFVHHIRVHSAKKFFVEESAEKQAKARESGSSTAEEGDFSKGPIRCDRCGYNTNRYDHYTAHLKHHTRAGDNERVYKCIICTYTTVSEYHWRKHLRNHFPRKVYTCGKCNYFSDRKNNYVQHVRTHTGERPYKCELCPYSSSQKTHLTRHMRTHSGEKPFKCDQCSYVASNQHEVTRHARQVHNGPKPLNCPHCDYKTADRSNFKKHVELHVNPRQFNCPVCDYAASKKCNLQYHFKSKHPTCPNKTMGSGGGGSGGGGSRADALDDFDLDMLGSDALDDFDLDMLGSDALDDFDLDMLGSDALDDFDLDMLYID

SEQ ID NO: 6 - DNA, 1032 bp, Artificial Sequence
  source 1..1032: mol_type = other DNA
atgcctaaaaagaaaagaaaggtgggttctggtaagaccaaaccctttcgctgtaagccatgccaatatgaagcagaatctgaagaacagtttgtgcatcacatcagagttcacagtgctaagaaattttttgtggaagagagtgcagagaagcaggcaaaagccagggaatctggctcttccactgcagaagagggagatttctccaagggccccattcgctgtgaccgctgcggctacaatactaatcgatatgatcactatacagcacacctgaaacaccacaccagagctggggataatgagcgagtctacaagtgtatcatttgcacatacacaacagtgagcgagtatcactggaggaaacatttaagaaaccattttccaaggaaagtatacacatgtggaaaatgcaactatttttcagacagaaaaaacaattatgttcagcatgttagaactcatacaggagaacgcccatataaatgtgaactttgtccttactcaagttctcagaagactcatctaactagacatatgcgtactcattcaggtgagaagccatttaaatgtgatcagtgcagttatgtggcctctaatcaacatgaagtaacccgccatgcaagacaggttcacaatgggcctaaacctcttaattgcccacactgtgattacaaaacagcagatagaagcaacttcaaaaaacatgtagagctacatgtgaacccacggcagttcaattgccctgtatgtgactatgcagcttccaagaagtgtaatctacagtatcacttcaaatctaagcatcctacttgtcctaataaaacaatgggtagtggcggtggtggttcaggaggcggcggaagccgcgccgacgcgctggacgatttcgatctcgacatgctgggttctgatgccctcgatgactttgacctggatatgttgggaagcgacgcattggatgactttgatctggacatgctcggctccgatgctctggacgatttcgatctcgatatgttatatatcgat

SEQ ID NO: 7 - protein, 55 aa, Artificial Sequence
RADALDDFDLDMLGSDALDDFDLDMLGSDALDDFDLDMLGSDALDDFDLDMLYID

SEQ ID NO: 8 - protein, 165 aa, Artificial Sequence
CGCGCCGACGCGCTGGACGATTTCGATCTCGACATGCTGGGTTCTGATGCCCTCGATGACTTTGACCTGGATATGTTGGGAAGCGACGCATTGGATGACTTTGATCTGGACATGCTCGGCTCCGATGCTCTGGACGATTTCGATCTCGATATGTTATATATCGAT

SEQ ID NO: 9 - protein, 680 aa, Artificial Sequence
MPKKKRKVGSGKTKPFRCKPCQYEAESEEQFVHHIRVHSAKKFFVEESAEKQAKARESGSSTAEEGDFSKGPIRCDRCGYNTNRYDHYTAHLKHHTRAGDNERVYKCIICTYTTVSEYHWRKHLRNHFPRKVYTCGKCNYFSDRKNNYVQHVRTHTGERPYKCELCPYSSSQKTHLTRHMRTHSGEKPFKCDQCSYVASNQHEVTRHARQVHNGPKPLNCPHCDYKTADRSNFKKHVELHVNPRQFNCPVCDYAASKKCNLQYHFKSKHPTCPNKTMGSGGGGSGGGGSRADALDDFDLDMLGSDALDDFDLDMLGSDALDDFDLDMLGSDALDDFDLDMLYIDDYKLGSGGGGSGGGGSPSGQISNQALALAPSSAPVLAQTMVPSSAMVPLAQPPAPAPVLTPGPPQSLSAPVPKSTQAGEGTLSEALLHLQFDADEDLGALLGNSTDPGVFTDLASVDNSEFQQLLNQGVSMSHSTAEPMLMEYPEAITRLVTGSQRPPDPAPTPLGTSGLPNGLSGDEDFSSIADMDFSALLSQISSSGQGGGGSGFSVDTSALLDLFSPSVTVPDMSLPDLDSSLASIQELLSPQEPPRPPEAENSSPDSGKQLVHYTAQPLFLLDPGSVDTGSNDLPVLFELGEGSYFSEGDGFAEDPTISLLTGSEPPKAKDPTVSPKKKRKV

SEQ ID NO: 10 - DNA, 2040 bp, Artificial Sequence
  source 1..2040: mol_type = other DNA
atgcctaaaaagaaaagaaaggtgggttctggtaagaccaaaccctttcgctgtaagccatgccaatatgaagcagaatctgaagaacagtttgtgcatcacatcagagttcacagtgctaagaaattttttgtggaagagagtgcagagaagcaggcaaaagccagggaatctggctcttccactgcagaagagggagatttctccaagggccccattcgctgtgaccgctgcggctacaatactaatcgatatgatcactatacagcacacctgaaacaccacaccagagctggggataatgagcgagtctacaagtgtatcatttgcacatacacaacagtgagcgagtatcactggaggaaacatttaagaaaccattttccaaggaaagtatacacatgtggaaaatgcaactatttttcagacagaaaaaacaattatgttcagcatgttagaactcatacaggagaacgcccatataaatgtgaactttgtccttactcaagttctcagaagactcatctaactagacatatgcgtactcattcaggtgagaagccatttaaatgtgatcagtgcagttatgtggcctctaatcaacatgaagtaacccgccatgcaagacaggttcacaatgggcctaaacctcttaattgcccacactgtgattacaaaacagcagatagaagcaacttcaaaaaacatgtagagctacatgtgaacccacggcagttcaattgccctgtatgtgactatgcagcttccaagaagtgtaatctacagtatcacttcaaatctaagcatcctacttgtcctaataaaacaatgggtagtggcggtggtggttcaggaggcggcggaagccgcgccgacgcgctggacgatttcgatctcgacatgctgggttctgatgccctcgatgactttgacctggatatgttgggaagcgacgcattggatgactttgatctggacatgctcggctccgatgctctggacgatttcgatctcgatatgttatatatcgatgattacaagcttggtagtggcggtggtggttcaggaggcggcggaagcccttcagggcagatcagcaaccaggccctggctctggcccctagctccgctccagtgctggcccagactatggtgccctctagtgctatggtgcctctggcccagccacctgctccagcccctgtgctgaccccaggaccaccccagtcactgagcgctccagtgcccaagtctacacaggccggcgaggggactctgagtgaagctctgctgcacctgcagttcgacgctgatgaggacctgggagctctgctggggaacagcaccgatcccggagtgttcacagatctggcctccgtggacaactctgagtttcagcagctgctgaatcagggcgtgtccatgtctcatagtacagccgaaccaatgctgatggagtaccccgaagccattacccggctggtgaccggcagccagcggccccccgaccccgctccaactcccctgggaaccagcggcctgcctaatgggctgtccggagatgaagacttctcaagcatcgctgatatggactttagtgccctgctgtcacagatttcctctagtgggcagggaggaggtggaagcggcttcagcgtggacaccagtgccctgctggacctgttcagcccctcggtgaccgtgcccgacatgagcctgcctgaccttgacagcagcctggccagtatccaagagctcctgtctccccaggagccccccaggcctcccgaggcagagaacagcagcccggattcagggaagcagctggtgcactacacagcgcagccgctgttcctgctggaccccggctccgtggacaccgggagcaacgacctgccggtgctgtttgagctgggagagggctcctacttctccgaaggggacggcttcgccgaggaccccaccatctccctgctgacaggctcggagcctcccaaagccaaggaccccactgtctcccccaagaagaagcgcaaggtg

SEQ ID NO: 11 - protein, 313 aa, Artificial Sequence
PSGQISNQALALAPSSAPVLAQTMVPSSAMVPLAQPPAPAPVLTPGPPQSLSAPVPKSTQAGEGTLSEALLHLQFDADEDLGALLGNSTDPGVFTDLASVDNSEFQQLLNQGVSMSHSTAEPMLMEYPEAITRLVTGSQRPPDPAPTPLGTSGLPNGLSGDEDFSSIADMDFSALLSQISSSGQGGGGSGFSVDTSALLDLFSPSVTVPDMSLPDLDSSLASIQELLSPQEPPRPPEAENSSPDSGKQLVHYTAQPLFLLDPGSVDTGSNDLPVLFELGEGSYFSEGDGFAEDPTISLLTGSEPPKAKDPTVS

SEQ ID NO: 12 - DNA, 939 bp, Artificial Sequence
  source 1..939: mol_type = other DNA
ccttcagggcagatcagcaaccaggccctggctctggcccctagctccgctccagtgctggcccagactatggtgccctctagtgctatggtgcctctggcccagccacctgctccagcccctgtgctgaccccaggaccaccccagtcactgagcgctccagtgcccaagtctacacaggccggcgaggggactctgagtgaagctctgctgcacctgcagttcgacgctgatgaggacctgggagctctgctggggaacagcaccgatcccggagtgttcacagatctggcctccgtggacaactctgagtttcagcagctgctgaatcagggcgtgtccatgtctcatagtacagccgaaccaatgctgatggagtaccccgaagccattacccggctggtgaccggcagccagcggccccccgaccccgctccaactcccctgggaaccagcggcctgcctaatgggctgtccggagatgaagacttctcaagcatcgctgatatggactttagtgccctgctgtcacagatttcctctagtgggcagggaggaggtggaagcggcttcagcgtggacaccagtgccctgctggacctgttcagcccctcggtgaccgtgcccgacatgagcctgcctgaccttgacagcagcctggccagtatccaagagctcctgtctccccaggagccccccaggcctcccgaggcagagaacagcagcccggattcagggaagcagctggtgcactacacagcgcagccgctgttcctgctggaccccggctccgtggacaccgggagcaacgacctgccggtgctgtttgagctgggagagggctcctacttctccgaaggggacggcttcgccgaggaccccaccatctccctgctgacaggctcggagcctcccaaagccaaggaccccactgtctcc

SEQ ID NO: 13 - protein, 18 aa, Artificial Sequence
KRTADGSEFESPKKKRKV

SEQ ID NO: 14 - DNA, 54 bp, Artificial Sequence
  source 1..54: mol_type = other DNA
aaacggacagccgatggcagcgagttcgagagccccaagaagaagagaaaggtg

SEQ ID NO: 15 - DNA, 798 bp, Artificial Sequence
  source 1..798: mol_type = other DNA
aagaccaagcccttcaggtgtaaaccctgccagtacgaggccgagtctgaggaacagtttgtccaccacatcagagtgcacagcgctaagaaattcttcgttgaggaatctgccgagaagcaggccaaggcccgggaaagcggctccagtacagccgaagagggcgacttcagcaagggccctatccggtgcgacagatgtggctataataccaacagatacgaccactacacagcgcacctgaagcaccacacccgggccggcgacaacgagagagtgtacaagtgcatcatctgcacctacaccacagtgtccgagtaccactggcggaaacatctcagaaaccactttccaagaaaggtgtacacctgcggcaagtgcaactacttcagcgaccggaagaacaactacgtgcagcacgtgcggacacacaccggcgagagaccttataagtgtgaactgtgcccttacagcagcagccagaaaactcacctgacccgccacatgagaacccatagcggagaaaagccatttaagtgcgaccagtgcagctacgtggccagcaatcaacacgaggtgaccagacacgccagacaggtgcacaacggccctaagcctctgaactgtccccactgcgactacaaaaccgccgatcggagcaacttcaagaaacacgtggaactgcacgtgaatcctagacagttcaactgccccgtgtgcgattacgccgcctccaagaagtgtaacctgcaataccacttcaagagcaagcatcctacatgccctaacaagaccatg

SEQ ID NO: 16 - protein, 112 aa, Artificial Sequence
MATQVMGQSSGGGGLFTSSGNIGMALPNDMYDLHDLSKAELAAPQLIMLANVALTGEVNGSCCDYLVGEERQMAELMPVGDNNFSDSEEGEGLEESADIKGEPHGLENMELR

SEQ ID NO: 17 - DNA, 336 bp, Artificial Sequence
  source 1..336: mol_type = other DNA
atggccacccaggtaatggggcagtcttctggaggaggagggctgtttaccagcagtggcaacattggaatggccctgcctaacgacatgtatgacttgcatgacctttccaaagctgaactggccgcacctcagcttattatgctggcaaatgtggccttaactggggaagtaaatggcagctgctgtgattacctggtcggtgaagaaagacagatggcagaactgatgccggttggggataacaacttttcagatagtgaagaaggagaaggacttgaagagtctgctgatataaaaggtgaacctcatggactggaaaacatggaactgaga

SEQ ID NO: 18 - protein, 91 aa, Artificial Sequence
MDEGIHSHEGSDLSDNMSEGSDDSGLHGARPVPQESSRKNAKEALAVKAAKGDFVCIFCDRSFRKGKDYSKHLNRHLVNVYYLEEAAQGQE

SEQ ID NO: 19 - DNA, 273 bp, Artificial Sequence
  source 1..273: mol_type = other DNA
atggatgaaggcatccacagccatgaaggaagtgacctaagtgacaacatgtcagagggtagtgatgattctggattgcatggggctcggccagttccacaagaatctagcagaaaaaatgcaaaggaagccttggcagtcaaagcggctaagggagattttgtttgtatcttctgtgatcgttctttcagaaagggaaaagattacagcaaacacctcaatcgccatttggttaatgtgtactatcttgaagaagcagctcaagggcaggag

SEQ ID NO: 20 - protein, 1097 aa, Artificial Sequence
MATQVMGQSSGGGGLFTSSGNIGMALPNDMYDLHDLSKAELAAPQLIMLANVALTGEVNGSCCDYLVGEERQMAELMPVGDNNFSDSEEGEGLEESADIKGEPHGLENMELRSLELSVVEPQPVFEASGAPDIYSSNKDLPPETPGAEDKGKSSKTKPFRCKPCQYEAESEEQFVHHIRVHSAKKFFVEESAEKQAKARESGSSTAEEGDFSKGPIRCDRCGYNTNRYDHYTAHLKHHTRAGDNERVYKCIICTYTTVSEYHWRKHLRNHFPRKVYTCGKCNYFSDRKNNYVQHVRTHTGERPYKCELCPYSSSQKTHLTRHMRTHSGEKPFKCDQCSYVASNQHEVTRHARQVHNGPKPLNCPHCDYKTADRSNFKKHVELHVNPRQFNCPVCDYAASKKCNLQYHFKSKHPTCPNKTMDVSKVKLKKTKKREADLPDNITNEKTEIEQTKIKGDVAGKKNEKSVKAEKRDVSKEKKPSNNVSVIQVTTRTRKSVTEVKEMDVHTGSNSEKFSKTKKSKRKLEVDSHSLHGPVNDEESSTKKKKKVESKSKNNSQEVPKGDSKVEENKKQNTCMKKSTKKKTLKNKSSKKSSKPPQKEPVEKGSAQMDPPQMGPAPTEAVQKGPVQVEPPPPMEHAQMEGAQIRPAPDEPVQMEVVQEGPAQKELLPPVEPAQMVGAQIVLAHMELPPPMETAQTEVAQMGPAPMEPAQMEVAQVESAPMQVVQKEPVQMELSPPMEVVQKEPVQIELSPPMEVVQKEPVKIELSPPIEVVQKEPVQMELSPPMGVVQKEPAQREPPPPREPPLHMEPISKKPPLRKDKKEKSNMQSERARKEQVLIEVGLVPVKDSWLLKESVSTEDLSPPSPPLPKENLREEASGDQKLLNTGEGNKEAPLQKVGAEEADESLPGLAANINESTHISSSGQNLNTPEGETLNGKHQTDSIVCEMKMDTDQNTRENLTGINSTVEEPVSPMLPPSAVEEREAVSKTALASPPATMAANESQEIDEDEGIHSHEGSDLSDNMSEGSDDSGLHGARPVPQESSRKNAKEALAVKAAKGDFVCIFCDRSFRKGKDYSKHLNRHLVNVYYLEEAAQGQE

SEQ ID NO: 21 - protein, 1054 aa, Artificial Sequence
MAKRNYILGLAIGITSVGYGIIDYETRDVIDAGVRLFKEANVENNEGRRSKRGARRLKRRRRHRIQRVKKLLFDYNLLTDHSELSGINPYEARVKGLSQKLSEEEFSAALLHLAKRRGVHNVNEVEEDTGNELSTKEQISRNSKALEEKYVAELQLERLKKDGEVRGSINRFKTSDYVKEAKQLLKVQKAYHQLDQSFIDTYIDLLETRRTYYEGPGEGSPFGWKDIKEWYEMLMGHCTYFPEELRSVKYAYNADLYNALNDLNNLVITRDENEKLEYYEKFQIIENVFKQKKKPTLKQIAKEILVNEEDIKGYRVTSTGKPEFTNLKVYHDIKDITARKEIIENAELLDQIAKILTIYQSSEDIQEELTNLNSELTQEEIEQISNLKGYTGTHNLSLKAINLILDELWHTNDNQIAIFNRLKLVPKKVDLSQQKEIPTTLVDDFILSPVVKRSFIQSIKVINAIIKKYGLPNDIIIELAREKNSKDAQKMINEMQKRNRQTNERIEEIIRTTGKENAKYLIEKIKLHDMQEGKCLYSLEAIPLEDLLNNPFNYEVDHIIPRSVSFDNSFNNKVLVKQEEASKKGNRTPFQYLSSSDSKISYETFKKHILNLAKGKGRISKTKKEYLLEERDINRFSVQKDFINRNLVDTRYATRGLMNLLRSYFRVNNLDVKVKSINGGFTSFLRRKWKFKKERNKGYKHHAEDALIIANADFIFKEWKKLDKAKKVMENQMFEEKQAESMPEIETEQEYKEIFITPHQIKHIKDFKDYKYSHRVDKKPNRKLINDTLYSTRKDDKGNTLIVNNLNGLYDKDNDKLKKLINKSPEKLLMYHHDPQTYQKLKLIMEQYGDEKNPLYKYYEETGNYLTKYSKKDNGPVIKKIKYYGNKLNAHLDITDDYPNSRNKVVKLSLKPYRFDVYLDNGVYKFVTVKNLDVIKKENYYEVNSKCYEEAKKLKKISNQAEFIASFYKNDLIKINGELYRVIGVNNDLLNRIEVNMIDITYREYLENMNDKRPPHIIKTIASKTQSIKKYSTDILGNLYEVKSKKHPQIIKKG

SEQ ID NO: 22 - protein, 1368 aa, Artificial Sequence
MDKKYSIGLAIGTNSVGWAVITDEYKVPSKKFKVLGNTDRHSIKKNLIGALLFDSGETAEATRLKRTARRRYTRRKNRICYLQEIFSNEMAKVDDSFFHRLEESFLVEEDKKHERHPIFGNIVDEVAYHEKYPTIYHLRKKLVDSTDKADLRLIYLALAHMIKFRGHFLIEGDLNPDNSDVDKLFIQLVQTYNQLFEENPINASGVDAKAILSARLSKSRRLENLIAQLPGEKKNGLFGNLIALSLGLTPNFKSNFDLAEDAKLQLSKDTYDDDLDNLLAQIGDQYADLFLAAKNLSDAILLSDILRVNTEITKAPLSASMIKRYDEHHQDLTLLKALVRQQLPEKYKEIFFDQSKNGYAGYIDGGASQEEFYKFIKPILEKMDGTEELLVKLNREDLLRKQRTFDNGSIPHQIHLGELHAILRRQEDFYPFLKDNREKIEKILTFRIPYYVGPLARGNSRFAWMTRKSEETITPWNFEEVVDKGASAQSFIERMTNFDKNLPNEKVLPKHSLLYEYFTVYNELTKVKYVTEGMRKPAFLSGEQKKAIVDLLFKTNRKVTVKQLKEDYFKKIECFDSVEISGVEDRFNASLGTYHDLLKIIKDKDFLDNEENEDILEDIVLTLTLFEDREMIEERLKTYAHLFDDKVMKQLKRRRYTGWGRLSRKLINGIRDKQSGKTILDFLKSDGFANRNFMQLIHDDSLTFKEDIQKAQVSGQGDSLHEHIANLAGSPAIKKGILQTVKVVDELVKVMGRHKPENIVIEMARENQTTQKGQKNSRERMKRIEEGIKELGSQILKEHPVENTQLQNEKLYLYYLQNGRDMYVDQELDINRLSDYDVDAIVPQSFLKDDSIDNKVLTRSDKNRGKSDNVPSEEVVKKMKNYWRQLLNAKLITQRKFDNLTKAERGGLSELDKAGFIKRQLVETRQITKHVAQILDSRMNTKYDENDKLIREVKVITLKSKLVSDFRKDFQFYKVREINNYHHAHDAYLNAVVGTALIKKYPKLESEFVYGDYKVYDVRKMIAKSEQEIGKATAKYFFYSNIMNFFKTEITLANGEIRKRPLIETNGETGEIVWDKGRDFATVRKVLSMPQVNIVKKTEVQTGGFSKESILPKRNSDKLIARKKDWDPKKYGGFDSPTVAYSVLVVAKVEKGKSKKLKSVKELLGITIMERSSFEKNPIDFLEAKGYKEVKKDLIIKLPKYSLFELENGRKRMLASAGELQKGNELALPSKYVNFLYLASHYEKLKGSPEDNEQKQLFVEQHKHYLDEIIEQISEFSKRVILADANLDKVLSAYNKHRDKPIREQAENIIHLFTLTNLGAPAAFKYFDTTIDRKRYTSTKEVLDATLIHQSITGLYETRIDLSQLGGD

SEQ ID NO: 23 - protein, 1519 aa, Artificial Sequence
MKRTADGSEFESPKKKRKVMDKKYSIGLAIGTNSVGWAVITDEYKVPSKKFKVLGNTDRHSIKKNLIGALLFDSGETAEATRLKRTARRRYTRRKNRICYLQEIFSNEMAKVDDSFFHRLEESFLVEEDKKHERHPIFGNIVDEVAYHEKYPTIYHLRKKLVDSTDKADLRLIYLALAHMIKFRGHFLIEGDLNPDNSDVDKLFIQLVQTYNQLFEENPINASGVDAKAILSARLSKSRRLENLIAQLPGEKKNGLFGNLIALSLGLTPNFKSNFDLAEDAKLQLSKDTYDDDLDNLLAQIGDQYADLFLAAKNLSDAILLSDILRVNTEITKAPLSASMIKRYDEHHQDLTLLKALVRQQLPEKYKEIFFDQSKNGYAGYIDGGASQEEFYKFIKPILEKMDGTEELLVKLNREDLLRKQRTFDNGSIPHQIHLGELHAILRRQEDFYPFLKDNREKIEKILTFRIPYYVGPLARGNSRFAWMTRKSEETITPWNFEEVVDKGASAQSFIERMTNFDKNLPNEKVLPKHSLLYEYFTVYNELTKVKYVTEGMRKPAFLSGEQKKAIVDLLFKTNRKVTVKQLKEDYFKKIECFDSVEISGVEDRFNASLGTYHDLLKIIKDKDFLDNEENEDILEDIVLTLTLFEDREMIEERLKTYAHLFDDKVMKQLKRRRYTGWGRLSRKLINGIRDKQSGKTILDFLKSDGFANRNFMQLIHDDSLTFKEDIQKAQVSGQGDSLHEHIANLAGSPAIKKGILQTVKVVDELVKVMGRHKPENIVIEMARENQTTQKGQKNSRERMKRIEEGIKELGSQILKEHPVENTQLQNEKLYLYYLQNGRDMYVDQELDINRLSDYDVDAIVPQSFLKDDSIDNKVLTRSDKNRGKSDNVPSEEVVKKMKNYWRQLLNAKLITQRKFDNLTKAERGGLSELDKAGFIKRQLVETRQITKHVAQILDSRMNTKYDENDKLIREVKVITLKSKLVSDFRKDFQFYKVREINNYHHAHDAYLNAVVGTALIKKYPKLESEFVYGDYKVYDVRKMIAKSEQEIGKATAKYFFYSNIMNFFKTEITLANGEIRKRPLIETNGETGEIVWDKGRDFATVRKVLSMPQVNIVKKTEVQTGGFSKESILPKRNSDKLIARKKDWDPKKYGGFDSPTVAYSVLVVAKVEKGKSKKLKSVKELLGITIMERSSFEKNPIDFLEAKGYKEVKKDLIIKLPKYSLFELENGRKRMLASAGELQKGNELALPSKYVNFLYLASHYEKLKGSPEDNEQKQLFVEQHKHYLDEIIEQISEFSKRVILADANLDKVLSAYNKHRDKPIREQAENIIHLFTLTNLGAPAAFKYFDTTIDRKRYTSTKEVLDATLIHQSITGLYETRIDLSQLGGDAKRTADGSEFESPKKKRKVAAADYKDDMGRVTFEDVTVNFTQGEWQRLNPEQRNLYRDVMLENYSNLVSVGQGETTKPDVILRLEQGKEPWLEEEEVLGSGRAEKNGDIGGQIWKPKDVKESLADYKDDDDK

SEQ ID NO: 24 - protein, 1407 aa, Artificial Sequence
MPKKKRKVGIHGVPAAKRNYILGLAIGITSVGYGIIDYETRDVIDAGVRLFKEANVENNEGRRSKRGARRLKRRRRHRIQRVKKLLFDYNLLTDHSELSGINPYEARVKGLSQKLSEEEFSAALLHLAKRRGVHNVNEVEEDTGNELSTKEQISRNSKALEEKYVAELQLERLKKDGEVRGSINRFKTSDYVKEAKQLLKVQKAYHQLDQSFIDTYIDLLETRRTYYEGPGEGSPFGWKDIKEWYEMLMGHCTYFPEELRSVKYAYNADLYNALNDLNNLVITRDENEKLEYYEKFQIIENVFKQKKKPTLKQIAKEILVNEEDIKGYRVTSTGKPEFTNLKVYHDIKDITARKEIIENAELLDQIAKILTIYQSSEDIQEELTNLNSELTQEEIEQISNLKGYTGTHNLSLKAINLILDELWHTNDNQIAIFNRLKLVPKKVDLSQQKEIPTTLVDDFILSPVVKRSFIQSIKVINAIIKKYGLPNDIIIELAREKNSKDAQKMINEMQKRNRQTNERIEEIIRTTGKENAKYLIEKIKLHDMQEGKCLYSLEAIPLEDLLNNPFNYEVDHIIPRSVSFDNSFNNKVLVKQEEASKKGNRTPFQYLSSSDSKISYETFKKHILNLAKGKGRISKTKKEYLLEERDINRFSVQKDFINRNLVDTRYATRGLMNLLRSYFRVNNLDVKVKSINGGFTSFLRRKWKFKKERNKGYKHHAEDALIIANADFIFKEWKKLDKAKKVMENQMFEEKQAESMPEIETEQEYKEIFITPHQIKHIKDFKDYKYSHRVDKKPNRKLINDTLYSTRKDDKGNTLIVNNLNGLYDKDNDKLKKLINKSPEKLLMYHHDPQTYQKLKLIMEQYGDEKNPLYKYYEETGNYLTKYSKKDNGPVIKKIKYYGNKLNAHLDITDDYPNSRNKVVKLSLKPYRFDVYLDNGVYKFVTVKNLDVIKKENYYEVNSKCYEEAKKLKKISNQAEFIASFYKNDLIKINGELYRVIGVNNDLLNRIEVNMIDITYREYLENMNDKRPPHIIKTIASKTQSIKKYSTDILGNLYEVKSKKHPQIIKKGKRPAATKKAGQAKKKKGSGSGGGGSGGGGSMGRVTFEDVTVNFTQGEWQRLNPEQRNLYRDVMLENYSNLVSVGQGETTKPDVILRLEQGKEPWLEEEEVLGSGRAEKNGDIGGQIWKPKDVKESLGGGGSMGRVTFEDVTVNFTQGEWQRLNPEQRNLYRDVMLENYSNLVSVGQGETTKPDVILRLEQGKEPWLEEEEVLGSGRAEKNGDIGGQIWKPKDVKESLGGGGSMGRVTFEDVTVNFTQGEWQRLNPEQRNLYRDVMLENYSNLVSVGQGETTKPDVILRLEQGKEPWLEEEEVLGSGRAEKNGDIGGQIWKPKDVKESLAAADYKDDDDK

SEQ ID NO: 25 - protein, 1455 aa, Artificial Sequence
MPKKKRKVGIHGVPAAKRNYILGLAIGITSVGYGIIDYETRDVIDAGVRLFKEANVENNEGRRSKRGARRLKRRRRHRIQRVKKLLFDYNLLTDHSELSGINPYEARVKGLSQKLSEEEFSAALLHLAKRRGVHNVNEVEEDTGNELSTKEQISRNSKALEEKYVAELQLERLKKDGEVRGSINRFKTSDYVKEAKQLLKVQKAYHQLDQSFIDTYIDLLETRRTYYEGPGEGSPFGWKDIKEWYEMLMGHCTYFPEELRSVKYAYNADLYNALNDLNNLVITRDENEKLEYYEKFQIIENVFKQKKKPTLKQIAKEILVNEEDIKGYRVTSTGKPEFTNLKVYHDIKDITARKEIIENAELLDQIAKILTIYQSSEDIQEELTNLNSELTQEEIEQISNLKGYTGTHNLSLKAINLILDELWHTNDNQIAIFNRLKLVPKKVDLSQQKEIPTTLVDDFILSPVVKRSFIQSIKVINAIIKKYGLPNDIIIELAREKNSKDAQKMINEMQKRNRQTNERIEEIIRTTGKENAKYLIEKIKLHDMQEGKCLYSLEAIPLEDLLNNPFNYEVDHIIPRSVSFDNSFNNKVLVKQEEASKKGNRTPFQYLSSSDSKISYETFKKHILNLAKGKGRISKTKKEYLLEERDINRFSVQKDFINRNLVDTRYATRGLMNLLRSYFRVNNLDVKVKSINGGFTSFLRRKWKFKKERNKGYKHHAEDALIIANADFIFKEWKKLDKAKKVMENQMFEEKQAESMPEIETEQEYKEIFITPHQIKHIKDFKDYKYSHRVDKKPNRKLINDTLYSTRKDDKGNTLIVNNLNGLYDKDNDKLKKLINKSPEKLLMYHHDPQTYQKLKLIMEQYGDEKNPLYKYYEETGNYLTKYSKKDNGPVIKKIKYYGNKLNAHLDITDDYPNSRNKVVKLSLKPYRFDVYLDNGVYKFVTVKNLDVIKKENYYEVNSKCYEEAKKLKKISNQAEFIASFYKNDLIKINGELYRVIGVNNDLLNRIEVNMIDITYREYLENMNDKRPPHIIKTIASKTQSIKKYSTDILGNLYEVKSKKHPQIIKKGKRPAATKKAGQAKKKKGSMATQVMGQSSGGGGLFTSSGNIGMALPNDMYDLHDLSKAELAAPQLIMLANVALTGEVNGSCCDYLVGEERQMAELMPVGDNNFSDSEEGEGLEESADIKGEPHGLENMELRGGGGSMATQVMGQSSGGGGLFTSSGNIGMALPNDMYDLHDLSKAELAAPQLIMLANVALTGEVNGSCCDYLVGEERQMAELMPVGDNNFSDSEEGEGLEESADIKGEPHGLENMELRGGGGSMATQVMGQSSGGGGLFTSSGNIGMALPNDMYDLHDLSKAELAAPQLIMLANVALTGEVNGSCCDYLVGEERQMAELMPVGDNNFSDSEEGEGLEESADIKGEPHGLENMELRGSGGGGSGGGGSAAADYKDDDDK

SEQ ID NO: 26 - protein, 1461 aa, Artificial Sequence
MPKKKRKVGIHGVPAKKKKGSMATQVMGQSSGGGGLFTSSGNIGMALPNDMYDLHDLSKAELAAPQLIMLANVALTGEVNGSCCDYLVGEERQMAELMPVGDNNFSDSEEGEGLEESADIKGEPHGLENMELRGGGGSMATQVMGQSSGGGGLFTSSGNIGMALPNDMYDLHDLSKAELAAPQLIMLANVALTGEVNGSCCDYLVGEERQMAELMPVGDNNFSDSEEGEGLEESADIKGEPHGLENMELRGGGGSMATQVMGQSSGGGGLFTSSGNIGMALPNDMYDLHDLSKAELAAPQLIMLANVALTGEVNGSCCDYLVGEERQMAELMPVGDNNFSDSEEGEGLEESADIKGEPHGLENMELRGSGGGGSGGGGSAKRNYILGLAIGITSVGYGIIDYETRDVIDAGVRLFKEANVENNEGRRSKRGARRLKRRRRHRIQRVKKLLFDYNLLTDHSELSGINPYEARVKGLSQKLSEEEFSAALLHLAKRRGVHNVNEVEEDTGNELSTKEQISRNSKALEEKYVAELQLERLKKDGEVRGSINRFKTSDYVKEAKQLLKVQKAYHQLDQSFIDTYIDLLETRRTYYEGPGEGSPFGWKDIKEWYEMLMGHCTYFPEELRSVKYAYNADLYNALNDLNNLVITRDENEKLEYYEKFQIIENVFKQKKKPTLKQIAKEILVNEEDIKGYRVTSTGKPEFTNLKVYHDIKDITARKEIIENAELLDQIAKILTIYQSSEDIQEELTNLNSELTQEEIEQISNLKGYTGTHNLSLKAINLILDELWHTNDNQIAIFNRLKLVPKKVDLSQQKEIPTTLVDDFILSPVVKRSFIQSIKVINAIIKKYGLPNDIIIELAREKNSKDAQKMINEMQKRNRQTNERIEEIIRTTGKENAKYLIEKIKLHDMQEGKCLYSLEAIPLEDLLNNPFNYEVDHIIPRSVSFDNSFNNKVLVKQEEASKKGNRTPFQYLSSSDSKISYETFKKHILNLAKGKGRISKTKKEYLLEERDINRFSVQKDFINRNLVDTRYATRGLMNLLRSYFRVNNLDVKVKSINGGFTSFLRRKWKFKKERNKGYKHHAEDALIIANADFIFKEWKKLDKAKKVMENQMFEEKQAESMPEIETEQEYKEIFITPHQIKHIKDFKDYKYSHRVDKKPNRKLINDTLYSTRKDDKGNTLIVNNLNGLYDKDNDKLKKLINKSPEKLLMYHHDPQTYQKLKLIMEQYGDEKNPLYKYYEETGNYLTKYSKKDNGPVIKKIKYYGNKLNAHLDITDDYPNSRNKVVKLSLKPYRFDVYLDNGVYKFVTVKNLDVIKKENYYEVNSKCYEEAKKLKKISNQAEFIASFYKNDLIKINGELYRVIGVNNDLLNRIEVNMIDITYREYLENMNDKRPPHIIKTIASKTQSIKKYSTDILGNLYEVKSKKHPQIIKKGKRPAATKKAGQAKKKKGSAAADYKDDDDK

SEQ ID NO: 27 - protein, 1757 aa, Artificial Sequence
MPKKKRKVGIHGVPAKKKKGSMATQVMGQSSGGGGLFTSSGNIGMALPNDMYDLHDLSKAELAAPQLIMLANVALTGEVNGSCCDYLVGEERQMAELMPVGDNNFSDSEEGEGLEESADIKGEPHGLENMELRGGGGSMATQVMGQSSGGGGLFTSSGNIGMALPNDMYDLHDLSKAELAAPQLIMLANVALTGEVNGSCCDYLVGEERQMAELMPVGDNNFSDSEEGEGLEESADIKGEPHGLENMELRGGGGSMATQVMGQSSGGGGLFTSSGNIGMALPNDMYDLHDLSKAELAAPQLIMLANVALTGEVNGSCCDYLVGEERQMAELMPVGDNNFSDSEEGEGLEESADIKGEPHGLENMELRGSGGGGSGGGGSAKRNYILGLAIGITSVGYGIIDYETRDVIDAGVRLFKEANVENNEGRRSKRGARRLKRRRRHRIQRVKKLLFDYNLLTDHSELSGINPYEARVKGLSQKLSEEEFSAALLHLAKRRGVHNVNEVEEDTGNELSTKEQISRNSKALEEKYVAELQLERLKKDGEVRGSINRFKTSDYVKEAKQLLKVQKAYHQLDQSFIDTYIDLLETRRTYYEGPGEGSPFGWKDIKEWYEMLMGHCTYFPEELRSVKYAYNADLYNALNDLNNLVITRDENEKLEYYEKFQIIENVFKQKKKPTLKQIAKEILVNEEDIKGYRVTSTGKPEFTNLKVYHDIKDITARKEIIENAELLDQIAKILTIYQSSEDIQEELTNLNSELTQEEIEQISNLKGYTGTHNLSLKAINLILDELWHTNDNQIAIFNRLKLVPKKVDLSQQKEIPTTLVDDFILSPVVKRSFIQSIKVINAIIKKYGLPNDIIIELAREKNSKDAQKMINEMQKRNRQTNERIEEIIRTTGKENAKYLIEKIKLHDMQEGKCLYSLEAIPLEDLLNNPFNYEVDHIIPRSVSFDNSFNNKVLVKQEEASKKGNRTPFQYLSSSDSKISYETFKKHILNLAKGKGRISKTKKEYLLEERDINRFSVQKDFINRNLVDTRYATRGLMNLLRSYFRVNNLDVKVKSINGGFTSFLRRKWKFKKERNKGYKHHAEDALIIANADFIFKEWKKLDKAKKVMENQMFEEKQAESMPEIETEQEYKEIFITPHQIKHIKDFKDYKYSHRVDKKPNRKLINDTLYSTRKDDKGNTLIVNNLNGLYDKDNDKLKKLINKSPEKLLMYHHDPQTYQKLKLIMEQYGDEKNPLYKYYEETGNYLTKYSKKDNGPVIKKIKYYGNKLNAHLDITDDYPNSRNKVVKLSLKPYRFDVYLDNGVYKFVTVKNLDVIKKENYYEVNSKCYEEAKKLKKISNQAEFIASFYKNDLIKINGELYRVIGVNNDLLNRIEVNMIDITYREYLENMNDKRPPHIIKTIASKTQSIKKYSTDILGNLYEVKSKKHPQIIKKGKRPAATKKAGQAKKKKGSAGSGGGGSGGGGSMDEGIHSHEGSDLSDNMSEGSDDSGLHGARPVPQESSRKNAKEALAVKAAKGDFVCIFCDRSFRKGKDYSKHLNRHLVNVYYLEEAAQGQEGGGGSMDEGIHSHEGSDLSDNMSEGSDDSGLHGARPVPQESSRKNAKEALAVKAAKGDFVCIFCDRSFRKGKDYSKHLNRHLVNVYYLEEAAQGQEGGGGSMDEGIHSHEGSDLSDNMSEGSDDSGLHGARPVPQESSRKNAKEALAVKAAKGDFVCIFCDRSFRKGKDYSKHLNRHLVNVYYLEEAAQGQEAAADYKDDDDK

SEQ ID NO: 28 - protein, 96 aa, Artificial Sequence
MGRVTFEDVTVNFTQGEWQRLNPEQRNLYRDVMLENYSNLVSVGQGETTKPDVILRLEQGKEPWLEEEEVLGSGRAEKNGDIGGQIWKPKDVKESL

SEQ ID NO: 29 - protein, 261 aa, Artificial Sequence
MDSSAVITQISKEEARGPLRGKGDQKSAASQKPRSRGILHSLFCCVCRDDGEALPAHSGAPLLVEENGAIPKQTPVQYLLPEAKAQDSDKICVVIDLDETLVHSSFKPVNNADFIIPVEIDGVVHQVYVLKRPHVDEFLQRMGELFECVLFTASLAKYADPVADLLDKWGAFRARLFRESCVFHRGNYVKDLSRLGRDLRRVLILDNSPASYVFHPDNAVPVASWFDNMSDTELHDLLPFFEQLSRVDDVYSVLRQPRPGS

SEQ ID NO: 30 - DNA, 786 bp, Artificial Sequence
  source 1..786: mol_type = other DNA
atggacagctcggccgtcattactcagatcagcaaggaggaggctcggggcccgctgcggggcaaaggtgaccagaagtcagcagcttcccagaagccccgaagccggggcatcctccactcactcttctgctgtgtctgccgggatgatggggaggccctgcctgctcacagcggggcgcccctgcttgtggaggagaatggcgccatccctaagcagaccccagtccaatacctgctccctgaggccaaggcccaggactcagacaagatctgcgtggtcatcgacctggacgagaccctggtgcacagctccttcaagccagtgaacaacgcggacttcatcatccctgtggagattgatggggtggtccaccaggtctacgtgttgaagcgtcctcacgtggatgagttcctgcagcgaatgggcgagctctttgaatgtgtgctgttcactgctagcctcgccaagtacgcagacccagtagctgacctgctggacaaatggggggccttccgggcccggctgtttcgagagtcctgcgtcttccaccgggggaactacgtgaaggacctgagccggttgggtcgagacctgcggcgggtgctcatcctggacaattcacctgcctcctatgtcttccatccagacaatgctgtaccggtggcctcgtggtttgacaacatgagtgacacagagctccacgacctcctccccttcttcgagcaactcagccgtgtggacgacgtgtactcagtgctcaggcagccacggccagggagctag

SEQ ID NO: 31 - DNA, 22 bp, Homo sapiens
  source 1..22: mol_type = genomic DNA
cgtgttcacagcggaccttgat

SEQ ID NO: 32 - DNA, 22 bp, Homo sapiens
  source 1..22: mol_type = genomic DNA
taaggcacgcggtgaatgccaa

SEQ ID NO: 33 - DNA, 109 bp, Homo sapiens
  source 1..109: mol_type = genomic DNA
atcaagattagaggctctgctctccgtgttcacagcggaccttgatttaatgtcatacaattaaggcacgcggtgaatgccaagagcggagcctacggctgcacttgaa

SEQ ID NO: 34 - DNA, 709 bp, Homo sapiens
  source 1..709: mol_type = genomic DNA
gggtaattaacttggatccacgccgtcatttgaaaactagatttataggcttatgtatgtttttaggcgtgtgctgtaaatggcatggagatatatgcatatgtatacgcaggcacacgcaccgtctacacttccacggaacagactaattaacagcggctctggcagatgtgtcagagatgagcagagacaggagctgggcttatgagttatgactctaggggtagagactcagagcggagagagggggatgggcagggagagaagagtggtaatcgcagtgggtcttatactttccggatcaagattagaggctctgctctccgtgttcacagcggaccttgatttaatgtcatacaattaaggcacgcggtgaatgccaagagcggagcctacggctgcacttgaaggacaccaaagcatctcagggtcagaaaggggaaaaagcaattgcagggaatttagggggtagtaaaaggaacccatctcttgccgcataaatgccccccacccccacccaggactgattctggaagcaacctagtgttcgaaagggaaaggctcctacttttccattacagccgcggaaatccgcaggcaaatctccgaggagaattttagggaagcttcattgacagctgtctggagagcagtagttcccgcctgtgcaaatattccagagagttaaatcatttagaaagcactagtt

SEQ ID NO: 35 - DNA, 23 bp, Homo sapiens
  source 1..23: mol_type = genomic DNA
tctttggttatctagctgtatga

SEQ ID NO: 36 - DNA, 22 bp, Homo sapiens
  source 1..22: mol_type = genomic DNA
ataaagctagataaccgaaagt

SEQ ID NO: 37 - DNA, 90 bp, Homo sapiens
  source 1..90: mol_type = genomic DNA
ggaggcccgtttctctctttggttatctagctgtatgagtgccacagagccgtcataaagctagataaccgaaagtagaaatgattctca

SEQ ID NO: 38 - DNA, 690 bp, Homo sapiens
  source 1..690: mol_type = genomic DNA
agcgctccgcgcgggtgccctacgtgagccccgggacgccgtcgaggcaggccggcagcgccggtgccaggacgcacggaacggggagcaggggagaaatgcgccgggagggcgagggaggaagggaactgggcgggggctgcgggcctaggtggcgggagtcagcgtgtgcgtgtgtctgtccatcccctctggctctccgcgtgcgccccaggatccgggcacggcgtccgctcaggctcccgcgctcggcaggcagcagcacgtggagcccacggcgcggcagcggcactggctaagggaggcccgtttctctctttggttatctagctgtatgagtgccacagagccgtcataaagctagataaccgaaagtagaaatgattctcacaacttctgcgtgcgagcgcccgccccaccgaccgccccggcccggcccgcaagagccagaggagccgagaggagcccagcgccggcccagcggactccagctcgacggagcggccgcgccccgaccaggtacctgacctcggctctctctctggggacacttgcagtgccagctttcccccagtcctcctctttcctggtcccccacccctatcccccagcgccggagcaggaaccccaaagtggagcgggccggggagagggagggggttggggttgcagaggggtcgctggaagggg

SEQ ID NO: 39 - DNA, 2209 bp, Homo sapiens
  source 1..2209: mol_type = other DNA
taatcccacctccctctctgtgctgggactcacagagggagacctcaggaggcagtctgtccatcacatgtccaaatgcagagcataccctgggctgggcgcagtggcgcacaactgtaattccagcactttgggaggctgatgtggaaggatcacttgagcccagaagttctagaccagcctgggcaacatggcaagaccctatctctacaaaaaaagttaaaaaatcagccacgtgtggtgacacacacctgtagtcccagctattcaggaggctgaggtgaggggatcacttaaggctgggaggttgaggctgcagtgagtcgtggttgcgccactgcactccagcctgggcaacagtgagaccctgtctcaaaagacaaaaaaaaaaaaaaaaaaaaaagaacatatcctggtgtggagtaggggacgctgctctgacagaggctcgggggcctgagctggctctgtgagctggggaggaggcagacagccaggccttgtctgcaagcagacctggcagcattgggctggccgccccccagggcctcctcttcatgcccagtgaatgactcaccttggcacagacacaatgttcggggtgggcacagtgcctgcttcccgccgcaccccagcccccctcaaatgccttccgagaagcccattgagcagggggcttgcattgcaccccagcctgacagcctggcatcttgggataaaagcagcacagccccctaggggctgcccttgctgtgtggcgccaccggcggtggagaacaaggctctattcagcctgtgcccaggaaaggggatcaggggatgcccaggcatggacagtgggtggcagggggggagaggagggctgtctgcttcccagaagtccaaggacacaaatgggtgaggggactgggcagggttctgaccctgtgggaccagagtggagggcgtagatggacctgaagtctccagggacaacagggcccaggtctcaggctcctagttgggcccagtggctccagcgtttccaaacccatccatccccagaggttcttcccatctctccaggctgatgtgtgggaactcgaggaaataaatctccagtgggagacggaggggtggccagggaaacggggcgctgcaggaataaagacgagccagcacagccagctcatgtgtaacggctttgtggagctgtcaaggcctggtctctgggagagaggcacagggaggccagacaaggaaggggtgacctggagggacagatccaggggctaaagtcctgataaggcaagagagtgccggccccctcttgccctatcaggacctccactgccacatagaggccatgattgacccttagacaaagggctggtgtccaatcccagcccccagccccagaactccagggaatgaatgggcagagagcaggaatgtgggacatctgtgttcaagggaaggactccaggagtctgctgggaatgaggcctagtaggaaatgaggtggcccttgagggtacagaacaggttcattcttcgccaaattcccagcaccttgcaggcacttacagctgagtgagataatgcctgggttatgaaatcaaaaagttggaaagcaggtcagaggtcatctggtacagcccttccttcccttttttttttttttttttgtgagacaaggtctctctctgttgcccaggctggagtggcgcaaacacagctcactgcagcctcaacctactgggctcaagcaatcctccagcctcagcctcccaaagtgctgggattacaagcatgagccaccccactcagccctttccttcctttttaattgatgcataataattgtaagtattcatcatggtccaaccaaccctttcttgacccaccttcctagagagagggtcctcttgcttcagcggtcagggccccagacccatggtctggctccaggtaccacctgcctcatgcaggagttggcgtgcccaggaagctctgcctctgggcacagtgacctcagtggggtgaggggagctctccccatagctgggctgcggcccaaccccaccccctcaggctatgccagggggtgttgccaggggcacccgggcatcgccagtctagcccactccttcataaagccctcgcatcccaggagcgagcagagccagagcaggttggagaggagacgcatcacctccgctgctcgcgg

SEQ ID NO: 40 - DNA, 681 bp, Homo sapiens
  source 1..681: mol_type = other DNA
aacatatcctggtgtggagtaggggacgctgctctgacagaggctcgggggcctgagctggctctgtgagctggggaggaggcagacagccaggccttgtctgcaagcagacctggcagcattgggctggccgccccccagggcctcctcttcatgcccagtgaatgactcaccttggcacagacacaatgttcggggtgggcacagtgcctgcttcccgccgcaccccagcccccctcaaatgccttccgagaagcccattgagcagggggcttgcattgcaccccagcctgacagcctggcatcttgggataaaagcagcacagccccctaggggctgcccttgctgtgtggcgccaccggcggtggagaacaaggctctattcagcctgtgcccaggaaaggggatcaggggatgcccaggcatggacagtgggtggcagggggggagaggagggctgtctgcttcccagaagtccaaggacacaaatgggtgaggggagagctctccccatagctgggctgcggcccaaccccaccccctcaggctatgccagggggtgttgccaggggcacccgggcatcgccagtctagcccactccttcataaagccctcgcatcccaggagcgagcagagccagagcaggttggagaggagacgcatcacctccgctgctcgc

SEQ ID NO: 41 - protein, 7 aa, Artificial Sequence
PKKKRKV

SEQ ID NO: 42 - protein, 16 aa, Artificial Sequence
KRPAATKKAGQAKKKK

SEQ ID NO: 43 - protein, 9 aa, Artificial Sequence
PAAKRVKLD

SEQ ID NO: 44 - protein, 11 aa, Artificial Sequence
RQRRNELKRSP

SEQ ID NO: 45 - protein, 38 aa, Artificial Sequence
NQSSNFGPMKGGNFGGRSSGPYGGGGQYFAKPRNQGGY

SEQ ID NO: 46 - protein, 42 aa, Artificial Sequence
RMRIZFKNKGKDTAELRRRRVEVSVELRKAKKDEQILKRRNV

SEQ ID NO: 47 - protein, 8 aa, Artificial Sequence
VSRKRPRP

SEQ ID NO: 48 - protein, 8 aa, Artificial Sequence
PPKKARED

SEQ ID NO: 49 - protein, 8 aa, Artificial Sequence
POPKKKPL

SEQ ID NO: 50 - protein, 12 aa, Artificial Sequence
SALIKKKKKMAP

SEQ ID NO: 51 - protein, 5 aa, Artificial Sequence
DRLRR

SEQ ID NO: 52 - protein, 7 aa, Artificial Sequence
PKQKKRK

SEQ ID NO: 53 - protein, 10 aa, Artificial Sequence
RKLKKKIKKL

SEQ ID NO: 54 - protein, 10 aa, Artificial Sequence
REKKKFLKRR

SEQ ID NO: 55 - protein, 20 aa, Artificial Sequence
KRKGDEVDGVDEVAKKKSKK

SEQ ID NO: 56 - protein, 17 aa, Artificial Sequence
RKCLQAGMNLEARKTKK

SEQ ID NO: 57 - protein, 11 aa, Artificial Sequence
LYPERLRRILT

SEQ ID NO: 58 - protein, 7 aa, Artificial Sequence
PKKKRKV